European Patent Specification EP 3 612 215 B1, published August 28, 2024. Title: COMPOSITIONS AND METHODS FOR TREATING LUNG INFLAMMATION. Applicant: ATYR PHARMA, INC. Mendlein, John D. Ogilvie, Kathleen. The sequence listing filed with the application follows.

SEQUENCE LISTING (233 sequences)

SEQ ID NO: 1 - protein, 509 aa, Homo sapiens
MAERAALEELVKLQGERVRGLKQQKASAELIEEEVAKLLKLKAQLGPDESKQKFVLKTPKGTRDYSPRQMAVREKVFDVIIRCFKRHGAEVIDTPVFELKETLMGKYGEDSKLIYDLKDQGGELLSLRYDLTVPFARYLAMNKLTNIKRYHIAKVYRRDNPAMTRGRYREFYQCDFDIAGNFDPMIPDAECLKIMCEILSSLQIGDFLVKVNDRRILDGMFAICGVSDSKFRTICSSVDKLDKVSWEEVKNEMVGEKGLAPEVADRIGDYVQQHGGVSLVEQLLQDPKLSQNKQALEGLGDLKLLFEYLTLFGIDDKISFDLSLARGLDYYTGVIYEAVLLQTPAQAGEEPLGVGSVAAGGRYDGLVGMFDPKGRKVPCVGLSIGVERIFSIVEQRLEALEEKIRTTETQVLVASAQKKLLEERLKLVSELWDAGIKAELLYKKNPKLLNQLQYCEEAGIPLVAIIGEQELKDGVIKLRSVTSREEVDVRREDLVEEIKRRTGQPLCIC

SEQ ID NO: 2 - protein, 500 aa, Homo sapiens
MAERAALEELVKLQGERVRGLKQQKASAELIEEEVAKLLKLKAQLGPDESKQKFVLKTPKGTRDYSPRQMAVREKVFDVIIRCFKRHGAEVIDTPVFELKETLMGKYGEDSKLIYDLKDQGGELLSLRYDLTVPFARYLAMNKLTNIKRYHIAKVYRRDNPAMTRGRYREFYQCDFDIAGNFDPMIPDAECLKIMCEILSSLQIGDFLVKVNDRRILDGMFAICGVSDSKFRTICSSVDKLDKVSWEEVKNEMVGEKGLAPEVADRIGDYVQQHGGVSLVEQLLQDPKLSQNKQALEGLGDLKLLFEYLTLFGIDDKISFDLSLARGLDYYTGVIYEAVLLQTPAQAGEEPLGVGSVAAGGRYDGLVGMFDPKGRKVPCVGLSIGVERIFSIVEQRLEALEEKIRTTETQVLVASAQKKLLEERLKLVSELWDAGIKAELLYKKNPKLLNQLQYCEEAGIPLVAIIGEQELKDGVIKLRSVTSREEVDVRREDLVEEIKR

SEQ ID NO: 3 - protein, 501 aa, Homo sapiens
MAERAALEELVKLQGERVRGLKQQKASAELIEEEVAKLLKLKAQLGPDESKQKFVLKTPKGTRDYSPRQMAVREKVFDVIIRCFKRHGAEVIDTPVFELKETLMGKYGEDSKLIYDLKDQGGELLSLRYDLTVPFARYLAMNKLTNIKRYHIAKVYRRDNPAMTRGRYREFYQCDFDIAGNFDPMIPDAECLKIMCEILSSLQIGDFLVKVNDRRILDGMFAICGVSDSKFRTICSSVDKLDKVSWEEVKNEMVGEKGLAPEVADRIGDYVQQHGGVSLVEQLLQDPKLSQNKQALEGLGDLKLLFEYLTLFGIDDKISFDLSLARGLDYYTGVIYEAVLLQTPAQAGEEPLGVGSVAAGGRYDGLVGMFDPKGRKVPCVGLSIGVERIFSIVEQRLEALEEKIRTTETQVLVASAQKKLLEERLKLVSELWDAGIKAELLYKKNPKLLNQLQYCEEAGIPLVAIIGEQELKDGVIKLRSVTSREEVDVRREDLVEEIKRR

SEQ ID NO: 4 - protein, 502 aa, Homo sapiens
MAERAALEELVKLQGERVRGLKQQKASAELIEEEVAKLLKLKAQLGPDESKQKFVLKTPKGTRDYSPRQMAVREKVFDVIIRCFKRHGAEVIDTPVFELKETLMGKYGEDSKLIYDLKDQGGELLSLRYDLTVPFARYLAMNKLTNIKRYHIAKVYRRDNPAMTRGRYREFYQCDFDIAGNFDPMIPDAECLKIMCEILSSLQIGDFLVKVNDRRILDGMFAICGVSDSKFRTICSSVDKLDKVSWEEVKNEMVGEKGLAPEVADRIGDYVQQHGGVSLVEQLLQDPKLSQNKQALEGLGDLKLLFEYLTLFGIDDKISFDLSLARGLDYYTGVIYEAVLLQTPAQAGEEPLGVGSVAAGGRYDGLVGMFDPKGRKVPCVGLSIGVERIFSIVEQRLEALEEKIRTTETQVLVASAQKKLLEERLKLVSELWDAGIKAELLYKKNPKLLNQLQYCEEAGIPLVAIIGEQELKDGVIKLRSVTSREEVDVRREDLVEEIKRRT

SEQ ID NO: 5 - protein, 503 aa, Homo sapiens
MAERAALEELVKLQGERVRGLKQQKASAELIEEEVAKLLKLKAQLGPDESKQKFVLKTPKGTRDYSPRQMAVREKVFDVIIRCFKRHGAEVIDTPVFELKETLMGKYGEDSKLIYDLKDQGGELLSLRYDLTVPFARYLAMNKLTNIKRYHIAKVYRRDNPAMTRGRYREFYQCDFDIAGNFDPMIPDAECLKIMCEILSSLQIGDFLVKVNDRRILDGMFAICGVSDSKFRTICSSVDKLDKVSWEEVKNEMVGEKGLAPEVADRIGDYVQQHGGVSLVEQLLQDPKLSQNKQALEGLGDLKLLFEYLTLFGIDDKISFDLSLARGLDYYTGVIYEAVLLQTPAQAGEEPLGVGSVAAGGRYDGLVGMFDPKGRKVPCVGLSIGVERIFSIVEQRLEALEEKIRTTETQVLVASAQKKLLEERLKLVSELWDAGIKAELLYKKNPKLLNQLQYCEEAGIPLVAIIGEQELKDGVIKLRSVTSREEVDVRREDLVEEIKRRTG

SEQ ID NO: 6 - protein, 504 aa, Homo sapiens
MAERAALEELVKLQGERVRGLKQQKASAELIEEEVAKLLKLKAQLGPDESKQKFVLKTPKGTRDYSPRQMAVREKVFDVIIRCFKRHGAEVIDTPVFELKETLMGKYGEDSKLIYDLKDQGGELLSLRYDLTVPFARYLAMNKLTNIKRYHIAKVYRRDNPAMTRGRYREFYQCDFDIAGNFDPMIPDAECLKIMCEILSSLQIGDFLVKVNDRRILDGMFAICGVSDSKFRTICSSVDKLDKVSWEEVKNEMVGEKGLAPEVADRIGDYVQQHGGVSLVEQLLQDPKLSQNKQALEGLGDLKLLFEYLTLFGIDDKISFDLSLARGLDYYTGVIYEAVLLQTPAQAGEEPLGVGSVAAGGRYDGLVGMFDPKGRKVPCVGLSIGVERIFSIVEQRLEALEEKIRTTETQVLVASAQKKLLEERLKLVSELWDAGIKAELLYKKNPKLLNQLQYCEEAGIPLVAIIGEQELKDGVIKLRSVTSREEVDVRREDLVEEIKRRTGQ

SEQ ID NO: 7 - protein, 505 aa, Homo sapiens
MAERAALEELVKLQGERVRGLKQQKASAELIEEEVAKLLKLKAQLGPDESKQKFVLKTPKGTRDYSPRQMAVREKVFDVIIRCFKRHGAEVIDTPVFELKETLMGKYGEDSKLIYDLKDQGGELLSLRYDLTVPFARYLAMNKLTNIKRYHIAKVYRRDNPAMTRGRYREFYQCDFDIAGNFDPMIPDAECLKIMCEILSSLQIGDFLVKVNDRRILDGMFAICGVSDSKFRTICSSVDKLDKVSWEEVKNEMVGEKGLAPEVADRIGDYVQQHGGVSLVEQLLQDPKLSQNKQALEGLGDLKLLFEYLTLFGIDDKISFDLSLARGLDYYTGVIYEAVLLQTPAQAGEEPLGVGSVAAGGRYDGLVGMFDPKGRKVPCVGLSIGVERIFSIVEQRLEALEEKIRTTETQVLVASAQKKLLEERLKLVSELWDAGIKAELLYKKNPKLLNQLQYCEEAGIPLVAIIGEQELKDGVIKLRSVTSREEVDVRREDLVEEIKRRTGQP

SEQ ID NO: 8 - protein, 506 aa, Homo sapiens
MAERAALEELVKLQGERVRGLKQQKASAELIEEEVAKLLKLKAQLGPDESKQKFVLKTPKGTRDYSPRQMAVREKVFDVIIRCFKRHGAEVIDTPVFELKETLMGKYGEDSKLIYDLKDQGGELLSLRYDLTVPFARYLAMNKLTNIKRYHIAKVYRRDNPAMTRGRYREFYQCDFDIAGNFDPMIPDAECLKIMCEILSSLQIGDFLVKVNDRRILDGMFAICGVSDSKFRTICSSVDKLDKVSWEEVKNEMVGEKGLAPEVADRIGDYVQQHGGVSLVEQLLQDPKLSQNKQALEGLGDLKLLFEYLTLFGIDDKISFDLSLARGLDYYTGVIYEAVLLQTPAQAGEEPLGVGSVAAGGRYDGLVGMFDPKGRKVPCVGLSIGVERIFSIVEQRLEALEEKIRTTETQVLVASAQKKLLEERLKLVSELWDAGIKAELLYKKNPKLLNQLQYCEEAGIPLVAIIGEQELKDGVIKLRSVTSREEVDVRREDLVEEIKRRTGQPL

SEQ ID NO: 9 - protein, 505 aa, Homo sapiens
AERAALEELVKLQGERVRGLKQQKASAELIEEEVAKLLKLKAQLGPDESKQKFVLKTPKGTRDYSPRQMAVREKVFDVIIRCFKRHGAEVIDTPVFELKETLMGKYGEDSKLIYDLKDQGGELLSLRYDLTVPFARYLAMNKLTNIKRYHIAKVYRRDNPAMTRGRYREFYQCDFDIAGNFDPMIPDAECLKIMCEILSSLQIGDFLVKVNDRRILDGMFAICGVSDSKFRTICSSVDKLDKVSWEEVKNEMVGEKGLAPEVADRIGDYVQQHGGVSLVEQLLQDPKLSQNKQALEGLGDLKLLFEYLTLFGIDDKISFDLSLARGLDYYTGVIYEAVLLQTPAQAGEEPLGVGSVAAGGRYDGLVGMFDPKGRKVPCVGLSIGVERIFSIVEQRLEALEEKIRTTETQVLVASAQKKLLEERLKLVSELWDAGIKAELLYKKNPKLLNQLQYCEEAGIPLVAIIGEQELKDGVIKLRSVTSREEVDVRREDLVEEIKRRTGQPL

SEQ ID NO: 10 - protein, 507 aa, Homo sapiens
MAERAALEELVKLQGERVRGLKQQKASAELIEEEVAKLLKLKAQLGPDESKQKFVLKTPKGTRDYSPRQMAVREKVFDVIIRCFKRHGAEVIDTPVFELKETLMGKYGEDSKLIYDLKDQGGELLSLRYDLTVPFARYLAMNKLTNIKRYHIAKVYRRDNPAMTRGRYREFYQCDFDIAGNFDPMIPDAECLKIMCEILSSLQIGDFLVKVNDRRILDGMFAICGVSDSKFRTICSSVDKLDKVSWEEVKNEMVGEKGLAPEVADRIGDYVQQHGGVSLVEQLLQDPKLSQNKQALEGLGDLKLLFEYLTLFGIDDKISFDLSLARGLDYYTGVIYEAVLLQTPAQAGEEPLGVGSVAAGGRYDGLVGMFDPKGRKVPCVGLSIGVERIFSIVEQRLEALEEKIRTTETQVLVASAQKKLLEERLKLVSELWDAGIKAELLYKKNPKLLNQLQYCEEAGIPLVAIIGEQELKDGVIKLRSVTSREEVDVRREDLVEEIKRRTGQPLC

SEQ ID NO: 11 - protein, 508 aa, Homo sapiens
MAERAALEELVKLQGERVRGLKQQKASAELIEEEVAKLLKLKAQLGPDESKQKFVLKTPKGTRDYSPRQMAVREKVFDVIIRCFKRHGAEVIDTPVFELKETLMGKYGEDSKLIYDLKDQGGELLSLRYDLTVPFARYLAMNKLTNIKRYHIAKVYRRDNPAMTRGRYREFYQCDFDIAGNFDPMIPDAECLKIMCEILSSLQIGDFLVKVNDRRILDGMFAICGVSDSKFRTICSSVDKLDKVSWEEVKNEMVGEKGLAPEVADRIGDYVQQHGGVSLVEQLLQDPKLSQNKQALEGLGDLKLLFEYLTLFGIDDKISFDLSLARGLDYYTGVIYEAVLLQTPAQAGEEPLGVGSVAAGGRYDGLVGMFDPKGRKVPCVGLSIGVERIFSIVEQRLEALEEKIRTTETQVLVASAQKKLLEERLKLVSELWDAGIKAELLYKKNPKLLNQLQYCEEAGIPLVAIIGEQELKDGVIKLRSVTSREEVDVRREDLVEEIKRRTGQPLCI

SEQ ID NO: 12 - protein, 48 aa, Homo sapiens
MAERAALEELVKLQGERVRGLKQQKASAELIEEEVAKLLKLKAQLGPD

SEQ ID NO: 13 - protein, 80 aa, Homo sapiens
MAERAALEELVKLQGERVRGLKQQKASAELIEEEVAKLLKLKAQLGPDESKQKFVLKTPKGTRDYSPRQMAVREKVFDVI

SEQ ID NO: 14 - protein, 79 aa, Homo sapiens
MAERAALEELVKLQGERVRGLKQQKASAELIEEEVAKLLKLKAQLGPDESKQKFVLKTPKGTRDYSPRQMAVREKVFDV

SEQ ID NO: 15 - protein, 78 aa, Homo sapiens
MAERAALEELVKLQGERVRGLKQQKASAELIEEEVAKLLKLKAQLGPDESKQKFVLKTPKGTRDYSPRQMAVREKVFD

SEQ ID NO: 16 - protein, 77 aa, Homo sapiens
MAERAALEELVKLQGERVRGLKQQKASAELIEEEVAKLLKLKAQLGPDESKQKFVLKTPKGTRDYSPRQMAVREKVF

SEQ ID NO: 17 - protein, 76 aa, Homo sapiens
MAERAALEELVKLQGERVRGLKQQKASAELIEEEVAKLLKLKAQLGPDESKQKFVLKTPKGTRDYSPRQMAVREKV

SEQ ID NO: 18 - protein, 75 aa, Homo sapiens
MAERAALEELVKLQGERVRGLKQQKASAELIEEEVAKLLKLKAQLGPDESKQKFVLKTPKGTRDYSPRQMAVREK

SEQ ID NO: 19 - protein, 74 aa, Homo sapiens
MAERAALEELVKLQGERVRGLKQQKASAELIEEEVAKLLKLKAQLGPDESKQKFVLKTPKGTRDYSPRQMAVRE

SEQ ID NO: 20 - protein, 73 aa, Homo sapiens
MAERAALEELVKLQGERVRGLKQQKASAELIEEEVAKLLKLKAQLGPDESKQKFVLKTPKGTRDYSPRQMAVR

SEQ ID NO: 21 - protein, 72 aa, Homo sapiens
MAERAALEELVKLQGERVRGLKQQKASAELIEEEVAKLLKLKAQLGPDESKQKFVLKTPKGTRDYSPRQMAV

SEQ ID NO: 22 - protein, 71 aa, Homo sapiens
MAERAALEELVKLQGERVRGLKQQKASAELIEEEVAKLLKLKAQLGPDESKQKFVLKTPKGTRDYSPRQMA

SEQ ID NO: 23 - protein, 70 aa, Homo sapiens
MAERAALEELVKLQGERVRGLKQQKASAELIEEEVAKLLKLKAQLGPDESKQKFVLKTPKGTRDYSPRQM

SEQ ID NO: 24 - protein, 69 aa, Homo sapiens
MAERAALEELVKLQGERVRGLKQQKASAELIEEEVAKLLKLKAQLGPDESKQKFVLKTPKGTRDYSPRQ

SEQ ID NO: 25 - protein, 68 aa, Homo sapiens
MAERAALEELVKLQGERVRGLKQQKASAELIEEEVAKLLKLKAQLGPDESKQKFVLKTPKGTRDYSPR

SEQ ID NO: 26 - protein, 67 aa, Homo sapiens
MAERAALEELVKLQGERVRGLKQQKASAELIEEEVAKLLKLKAQLGPDESKQKFVLKTPKGTRDYSP

SEQ ID NO: 27 - protein, 66 aa, Homo sapiens
MAERAALEELVKLQGERVRGLKQQKASAELIEEEVAKLLKLKAQLGPDESKQKFVLKTPKGTRDYS

SEQ ID NO: 28 - protein, 65 aa, Homo sapiens
MAERAALEELVKLQGERVRGLKQQKASAELIEEEVAKLLKLKAQLGPDESKQKFVLKTPKGTRDY

SEQ ID NO: 29 - protein, 64 aa, Homo sapiens
MAERAALEELVKLQGERVRGLKQQKASAELIEEEVAKLLKLKAQLGPDESKQKFVLKTPKGTRD

SEQ ID NO: 30 - protein, 63 aa, Homo sapiens
MAERAALEELVKLQGERVRGLKQQKASAELIEEEVAKLLKLKAQLGPDESKQKFVLKTPKGTR

SEQ ID NO: 31 - protein, 62 aa, Homo sapiens
MAERAALEELVKLQGERVRGLKQQKASAELIEEEVAKLLKLKAQLGPDESKQKFVLKTPKGT

SEQ ID NO: 32 - protein, 61 aa, Homo sapiens
MAERAALEELVKLQGERVRGLKQQKASAELIEEEVAKLLKLKAQLGPDESKQKFVLKTPKG

SEQ ID NO: 33 - protein, 60 aa, Homo sapiens
MAERAALEELVKLQGERVRGLKQQKASAELIEEEVAKLLKLKAQLGPDESKQKFVLKTPK

SEQ ID NO: 34 - protein, 59 aa, Homo sapiens
MAERAALEELVKLQGERVRGLKQQKASAELIEEEVAKLLKLKAQLGPDESKQKFVLKTP

SEQ ID NO: 35 - protein, 58 aa, Homo sapiens
MAERAALEELVKLQGERVRGLKQQKASAELIEEEVAKLLKLKAQLGPDESKQKFVLKT

SEQ ID NO: 36 - protein, 57 aa, Homo sapiens
MAERAALEELVKLQGERVRGLKQQKASAELIEEEVAKLLKLKAQLGPDESKQKFVLK

SEQ ID NO: 37 - protein, 56 aa, Homo sapiens
MAERAALEELVKLQGERVRGLKQQKASAELIEEEVAKLLKLKAQLGPDESKQKFVL

SEQ ID NO: 38 - protein, 55 aa, Homo sapiens
MAERAALEELVKLQGERVRGLKQQKASAELIEEEVAKLLKLKAQLGPDESKQKFV

SEQ ID NO: 39 - protein, 54 aa, Homo sapiens
MAERAALEELVKLQGERVRGLKQQKASAELIEEEVAKLLKLKAQLGPDESKQKF

SEQ ID NO: 40 - protein, 53 aa, Homo sapiens
MAERAALEELVKLQGERVRGLKQQKASAELIEEEVAKLLKLKAQLGPDESKQK

SEQ ID NO: 41 - protein, 52 aa, Homo sapiens
MAERAALEELVKLQGERVRGLKQQKASAELIEEEVAKLLKLKAQLGPDESKQ

SEQ ID NO: 42 - protein, 51 aa, Homo sapiens
MAERAALEELVKLQGERVRGLKQQKASAELIEEEVAKLLKLKAQLGPDESK

SEQ ID NO: 43 - protein, 50 aa, Homo sapiens
MAERAALEELVKLQGERVRGLKQQKASAELIEEEVAKLLKLKAQLGPDES

SEQ ID NO: 44 - protein, 49 aa, Homo sapiens
MAERAALEELVKLQGERVRGLKQQKASAELIEEEVAKLLKLKAQLGPDE

SEQ ID NO: 45 - protein, 48 aa, Homo sapiens; identical to SEQ ID NO: 12

SEQ ID NO: 46 - protein, 47 aa, Homo sapiens
MAERAALEELVKLQGERVRGLKQQKASAELIEEEVAKLLKLKAQLGP

SEQ ID NO: 47 - protein, 46 aa, Homo sapiens
MAERAALEELVKLQGERVRGLKQQKASAELIEEEVAKLLKLKAQLG

SEQ ID NO: 48 - protein, 45 aa, Homo sapiens
MAERAALEELVKLQGERVRGLKQQKASAELIEEEVAKLLKLKAQL

SEQ ID NO: 49 - protein, 44 aa, Homo sapiens
MAERAALEELVKLQGERVRGLKQQKASAELIEEEVAKLLKLKAQ

SEQ ID NO: 50 - protein, 43 aa, Homo sapiens
MAERAALEELVKLQGERVRGLKQQKASAELIEEEVAKLLKLKA

SEQ ID NO: 51 - protein, 42 aa, Homo sapiens
MAERAALEELVKLQGERVRGLKQQKASAELIEEEVAKLLKLK

SEQ ID NO: 52 - protein, 41 aa, Homo sapiens
MAERAALEELVKLQGERVRGLKQQKASAELIEEEVAKLLKL

SEQ ID NO: 53 - protein, 40 aa, Homo sapiens
MAERAALEELVKLQGERVRGLKQQKASAELIEEEVAKLLK

SEQ ID NO: 54 - protein, 79 aa, Homo sapiens
AERAALEELVKLQGERVRGLKQQKASAELIEEEVAKLLKLKAQLGPDESKQKFVLKTPKGTRDYSPRQMAVREKVFDVI

SEQ ID NO: 55 - protein, 78 aa, Homo sapiens
ERAALEELVKLQGERVRGLKQQKASAELIEEEVAKLLKLKAQLGPDESKQKFVLKTPKGTRDYSPRQMAVREKVFDVI

SEQ ID NO: 56 - protein, 77 aa, Homo sapiens
RAALEELVKLQGERVRGLKQQKASAELIEEEVAKLLKLKAQLGPDESKQKFVLKTPKGTRDYSPRQMAVREKVFDVI

SEQ ID NO: 57 - protein, 76 aa, Homo sapiens
AALEELVKLQGERVRGLKQQKASAELIEEEVAKLLKLKAQLGPDESKQKFVLKTPKGTRDYSPRQMAVREKVFDVI

SEQ ID NO: 58 - protein, 75 aa, Homo sapiens
ALEELVKLQGERVRGLKQQKASAELIEEEVAKLLKLKAQLGPDESKQKFVLKTPKGTRDYSPRQMAVREKVFDVI

SEQ ID NO: 59 - protein, 74 aa, Homo sapiens
LEELVKLQGERVRGLKQQKASAELIEEEVAKLLKLKAQLGPDESKQKFVLKTPKGTRDYSPRQMAVREKVFDVI

SEQ ID NO: 60 - protein, 73 aa, Homo sapiens
EELVKLQGERVRGLKQQKASAELIEEEVAKLLKLKAQLGPDESKQKFVLKTPKGTRDYSPRQMAVREKVFDVI

SEQ ID NO: 61 - protein, 72 aa, Homo sapiens
ELVKLQGERVRGLKQQKASAELIEEEVAKLLKLKAQLGPDESKQKFVLKTPKGTRDYSPRQMAVREKVFDVI

SEQ ID NO: 62 - protein, 71 aa, Homo sapiens
LVKLQGERVRGLKQQKASAELIEEEVAKLLKLKAQLGPDESKQKFVLKTPKGTRDYSPRQMAVREKVFDVI

SEQ ID NO: 63 - protein, 70 aa, Homo sapiens
VKLQGERVRGLKQQKASAELIEEEVAKLLKLKAQLGPDESKQKFVLKTPKGTRDYSPRQMAVREKVFDVI

SEQ ID NO: 64 - protein, 69 aa, Homo sapiens
KLQGERVRGLKQQKASAELIEEEVAKLLKLKAQLGPDESKQKFVLKTPKGTRDYSPRQMAVREKVFDVI

SEQ ID NO: 65 - protein, 68 aa, Homo sapiens
LQGERVRGLKQQKASAELIEEEVAKLLKLKAQLGPDESKQKFVLKTPKGTRDYSPRQMAVREKVFDVI

SEQ ID NO: 66 - protein, 67 aa, Homo sapiens
QGERVRGLKQQKASAELIEEEVAKLLKLKAQLGPDESKQKFVLKTPKGTRDYSPRQMAVREKVFDVI

SEQ ID NO: 67 - protein, 66 aa, Homo sapiens
GERVRGLKQQKASAELIEEEVAKLLKLKAQLGPDESKQKFVLKTPKGTRDYSPRQMAVREKVFDVI

SEQ ID NO: 68 - protein, 64 aa, Homo sapiens
RVRGLKQQKASAELIEEEVAKLLKLKAQLGPDESKQKFVLKTPKGTRDYSPRQMAVREKVFDVI

SEQ ID NO: 69 - protein, 63 aa, Homo sapiens
VRGLKQQKASAELIEEEVAKLLKLKAQLGPDESKQKFVLKTPKGTRDYSPRQMAVREKVFDVI

SEQ ID NO: 70 - protein, 62 aa, Homo sapiens
RGLKQQKASAELIEEEVAKLLKLKAQLGPDESKQKFVLKTPKGTRDYSPRQMAVREKVFDVI

SEQ ID NO: 71 - protein, 61 aa, Homo sapiens
GLKQQKASAELIEEEVAKLLKLKAQLGPDESKQKFVLKTPKGTRDYSPRQMAVREKVFDVI

SEQ ID NO: 72 - protein, 60 aa, Homo sapiens
LKQQKASAELIEEEVAKLLKLKAQLGPDESKQKFVLKTPKGTRDYSPRQMAVREKVFDVI

SEQ ID NO: 73 - protein, 59 aa, Homo sapiens
KQQKASAELIEEEVAKLLKLKAQLGPDESKQKFVLKTPKGTRDYSPRQMAVREKVFDVI

SEQ ID NO: 74 - protein, 58 aa, Homo sapiens
QQKASAELIEEEVAKLLKLKAQLGPDESKQKFVLKTPKGTRDYSPRQMAVREKVFDVI

SEQ ID NO: 75 - protein, 57 aa, Homo sapiens
QKASAELIEEEVAKLLKLKAQLGPDESKQKFVLKTPKGTRDYSPRQMAVREKVFDVI

SEQ ID NO: 76 - protein, 56 aa, Homo sapiens
KASAELIEEEVAKLLKLKAQLGPDESKQKFVLKTPKGTRDYSPRQMAVREKVFDVI

SEQ ID NO: 77 - protein, 55 aa, Homo sapiens
ASAELIEEEVAKLLKLKAQLGPDESKQKFVLKTPKGTRDYSPRQMAVREKVFDVI

SEQ ID NO: 78 - protein, 54 aa, Homo sapiens
SAELIEEEVAKLLKLKAQLGPDESKQKFVLKTPKGTRDYSPRQMAVREKVFDVI

SEQ ID NO: 79 - protein, 53 aa, Homo sapiens
AELIEEEVAKLLKLKAQLGPDESKQKFVLKTPKGTRDYSPRQMAVREKVFDVI

SEQ ID NO: 80 - protein, 52 aa, Homo sapiens
ELIEEEVAKLLKLKAQLGPDESKQKFVLKTPKGTRDYSPRQMAVREKVFDVI

SEQ ID NO: 81 - protein, 51 aa, Homo sapiens
LIEEEVAKLLKLKAQLGPDESKQKFVLKTPKGTRDYSPRQMAVREKVFDVI

SEQ ID NO: 82 - protein, 50 aa, Homo sapiens
IEEEVAKLLKLKAQLGPDESKQKFVLKTPKGTRDYSPRQMAVREKVFDVI

SEQ ID NO: 83 - protein, 49 aa, Homo sapiens
EEEVAKLLKLKAQLGPDESKQKFVLKTPKGTRDYSPRQMAVREKVFDVI

SEQ ID NO: 84 - protein, 48 aa, Homo sapiens
EEVAKLLKLKAQLGPDESKQKFVLKTPKGTRDYSPRQMAVREKVFDVI

SEQ ID NO: 85 - protein, 47 aa, Homo sapiens
EVAKLLKLKAQLGPDESKQKFVLKTPKGTRDYSPRQMAVREKVFDVI

SEQ ID NO: 86 - protein, 46 aa, Homo sapiens
VAKLLKLKAQLGPDESKQKFVLKTPKGTRDYSPRQMAVREKVFDVI

SEQ ID NO: 87 - protein, 45 aa, Homo sapiens
AKLLKLKAQLGPDESKQKFVLKTPKGTRDYSPRQMAVREKVFDVI

SEQ ID NO: 88 - protein, 44 aa, Homo sapiens
KLLKLKAQLGPDESKQKFVLKTPKGTRDYSPRQMAVREKVFDVI

SEQ ID NO: 89 - protein, 43 aa, Homo sapiens
LLKLKAQLGPDESKQKFVLKTPKGTRDYSPRQMAVREKVFDVI

SEQ ID NO: 90 - protein, 42 aa, Homo sapiens
LKLKAQLGPDESKQKFVLKTPKGTRDYSPRQMAVREKVFDVI

SEQ ID NO: 91 - protein, 41 aa, Homo sapiens
KLKAQLGPDESKQKFVLKTPKGTRDYSPRQMAVREKVFDVI

SEQ ID NO: 92 - protein, 40 aa, Homo sapiens
LKAQLGPDESKQKFVLKTPKGTRDYSPRQMAVREKVFDVI

SEQ ID NO: 93 - protein, 141 aa, Homo sapiens
MAERAALEELVKLQGERVRGLKQQKASAELIEEEVAKLLKLKAQLGPDESKQKFVLKTPKGTRDYSPRQMAVREKVFDVIIRCFKRHGAEVIDTPVFELKETLMGKYGEDSKLIYDLKDQGGELLSLRYDLTVPFARYLAM

SEQ ID NO: 94 - protein, 408 aa, Homo sapiens
MAERAALEELVKLQGERVRGLKQQKASAELIEEEVAKLLKLKAQLGPDESKQKFVLKTPKGTRDYSPRQMAVREKVFDVIIRCFKRHGAEVIDTPVFELKETLMGKYGEDSKLIYDLKDQGGELLSLRYDLTVPFARYLAMNKLTNIKRYHIAKVYRRDNPAMTRGRYREFYQCDFDIAGNFDPMIPDAECLKIMCEILSSLQIGDFLVKVNDRRILDGMFAICGVSDSKFRTICSSVDKLDKVSWEEVKNEMVGEKGLAPEVADRIGDYVQQHGGVSLVEQLLQDPKLSQNKQALEGLGDLKLLFEYLTLFGIDDKISFDLSLARGLDYYTGVIYEAVLLQTPAQAGEEPLGVGSVAAGGRYDGLVGMFDPKGRKVPCVGLSIGVERIFSIVEQRLEALEEKIRTTE

SEQ ID NO: 95 - protein, 113 aa, Homo sapiens
MAERAALEELVKLQGERVRGLKQQKASAELIEEEVAKLLKLKAQLGPDESKQKFVLKTPKGTRDYSPRQMAVREKVFDVIIRCFKRHGAEVIDTPVFELKETLMGKYGEDSKL

SEQ ID NO: 96 - protein, 60 aa, Homo sapiens; identical to SEQ ID NO: 33

SEQ ID NO: 97 - protein, 270 aa, Homo sapiens
MAERAALEELVKLQGERVRGLKQQKASAELIEEEVAKLLKLKAQLGPDESKQKFVLKTPKGTRDYSPRQMAVREKVFDVIIRCFKRHGAEVIDTPVFELKETLMGKYGEDSKLIYDLKDQGGELLSLRYDLTVPFARYLAMNKLTNIKRYHIAKVYRRDNPAMTRGRYREFYQCDFDIAGNFDPMIPDAECLKIMCEILSSLQIGDFLVKVNDRRILDGMFAICGVSDSKFRTICSSVDKLDKVGYPWWNSCSRILNYPKTSRPWRAWET

SEQ ID NO: 98 - protein, 105 aa, Homo sapiens
RTTETQVLVASAQKKLLEERLKLVSELWDAGIKAELLYKKNPKLLNQLQYCEEAGIPLVAIIGEQELKDGVIKLRSVTSREEVDVRREDLVEEIKRRTGQPLCIC

SEQ ID NO: 99 - protein, 395 aa, Homo sapiens
MAERAALEELVKLQGERVRGLKQQKASAELIEEEVAKLLKLKAQLGPDESKQKFVLKTPKDFDIAGNFDPMIPDAECLKIMCEILSSLQIGDFLVKVNDRRILDGMFAICGVSDSKFRTICSSVDKLDKVSWEEVKNEMVGEKGLAPEVADRIGDYVQQHGGVSLVEQLLQDPKLSQNKQALEGLGDLKLLFEYLTLFGIDDKISFDLSLARGLDYYTGVIYEAVLLQTPAQAGEEPLGVGSVAAGGRYDGLVGMFDPKGRKVPCVGLSIGVERIFSIVEQRLEALEEKIRTTETQVLVASAQKKLLEERLKLVSELWDAGIKAELLYKKNPKLLNQLQYCEEAGIPLVAIIGEQELKDGVIKLRSVTSREEVDVRREDLVEEIKRRTGQPLCIC

SEQ ID NO: 100 - protein, 359 aa, Homo sapiens
MAERAALEELVKLQGERVRGLKQQKASAELIEEEVAKLLKLKAQLGPDESKQKFVLKTPKVNDRRILDGMFAICGVSDSKFRTICSSVDKLDKVSWEEVKNEMVGEKGLAPEVADRIGDYVQQHGGVSLVEQLLQDPKLSQNKQALEGLGDLKLLFEYLTLFGIDDKISFDLSLARGLDYYTGVIYEAVLLQTPAQAGEEPLGVGSVAAGGRYDGLVGMFDPKGRKVPCVGLSIGVERIFSIVEQRLEALEEKIRTTETQVLVASAQKKLLEERLKLVSELWDAGIKAELLYKKNPKLLNQLQYCEEAGIPLVAIIGEQELKDGVIKLRSVTSREEVDVRREDLVEEIKRRTGQPLCIC

SEQ ID NO: 101 - protein, 399 aa, Homo sapiens
MAERAALEELVKLQGERVRGLKQQKASAELIEEEVAKLLKLKAQLGPDESKQKFVLKTPKGTRDYSPRQMAVREKVFDVIIRCFKRHGAEVIDTPVFELKVNDRRILDGMFAICGVSDSKFRTICSSVDKLDKVSWEEVKNEMVGEKGLAPEVADRIGDYVQQHGGVSLVEQLLQDPKLSQNKQALEGLGDLKLLFEYLTLFGIDDKISFDLSLARGLDYYTGVIYEAVLLQTPAQAGEEPLGVGSVAAGGRYDGLVGMFDPKGRKVPCVGLSIGVERIFSIVEQRLEALEEKIRTTETQVLVASAQKKLLEERLKLVSELWDAGIKAELLYKKNPKLLNQLQYCEEAGIPLVAIIGEQELKDGVIKLRSVTSREEVDVRREDLVEEIKRRTGQPLCIC

SEQ ID NO: 102 - protein, 473 aa, Homo sapiens
MAERAALEELVKLQGERVRGLKQQKASAELIEEEVAKLLKLKAQLGPDESKQKFVLKTPKGTRDYSPRQMAVREKVFDVIIRCFKRHGAEVIDTPVFELKETLMGKYGEDSKLIYDLKDQGGELLSLRYDLTVPFARYLAMNKLTNIKRYHIAKVYRRDNPAMTRGRYREFYQCVNDRRILDGMFAICGVSDSKFRTICSSVDKLDKVSWEEVKNEMVGEKGLAPEVADRIGDYVQQHGGVSLVEQLLQDPKLSQNKQALEGLGDLKLLFEYLTLFGIDDKISFDLSLARGLDYYTGVIYEAVLLQTPAQAGEEPLGVGSVAAGGRYDGLVGMFDPKGRKVPCVGLSIGVERIFSIVEQRLEALEEKIRTTETQVLVASAQKKLLEERLKLVSELWDAGIKAELLYKKNPKLLNQLQYCEEAGIPLVAIIGEQELKDGVIKLRSVTSREEVDVRREDLVEEIKRRTGQPLCIC

SEQ ID NO: 103 - protein, 469 aa, Homo sapiens
MAERAALEELVKLQGERVRGLKQQKASAELIEEEVAKLLKLKAQLGPDESKQKFVLKTPKETLMGKYGEDSKLIYDLKDQGGELLSLRYDLTVPFARYLAMNKLTNIKRYHIAKVYRRDNPAMTRGRYREFYQCDFDIAGNFDPMIPDAECLKIMCEILSSLQIGDFLVKVNDRRILDGMFAICGVSDSKFRTICSSVDKLDKVSWEEVKNEMVGEKGLAPEVADRIGDYVQQHGGVSLVEQLLQDPKLSQNKQALEGLGDLKLLFEYLTLFGIDDKISFDLSLARGLDYYTGVIYEAVLLQTPAQAGEEPLGVGSVAAGGRYDGLVGMFDPKGRKVPCVGLSIGVERIFSIVEQRLEALEEKIRTTETQVLVASAQKKLLEERLKLVSELWDAGIKAELLYKKNPKLLNQLQYCEEAGIPLVAIIGEQELKDGVIKLRSVTSREEVDVRREDLVEEIKRRTGQPLCIC

SEQ ID NO: 104 - protein, 435 aa, Homo sapiens
MAERAALEELVKLQGERVRGLKQQKASAELIEEEVAKLLKLKAQLGPDESKQKFVLKTPKGTRDYSPRQMAVREKVFDVIIRCFKRHGAEVIDTPVFELKDFDIAGNFDPMIPDAECLKIMCEILSSLQIGDFLVKVNDRRILDGMFAICGVSDSKFRTICSSVDKLDKVSWEEVKNEMVGEKGLAPEVADRIGDYVQQHGGVSLVEQLLQDPKLSQNKQALEGLGDLKLLFEYLTLFGIDDKISFDLSLARGLDYYTGVIYEAVLLQTPAQAGEEPLGVGSVAAGGRYDGLVGMFDPKGRKVPCVGLSIGVERIFSIVEQRLEALEEKIRTTETQVLVASAQKKLLEERLKLVSELWDAGIKAELLYKKNPKLLNQLQYCEEAGIPLVAIIGEQELKDGVIKLRSVTSREEVDVRREDLVEEIKRRTGQPLCIC

SEQ ID NO: 105 - protein, 171 aa, Homo sapiens
MAERAALEELVKLQGERVRGLKQQKASAELIEEEVAKLLKLKAQLGPDESKQKFVLKTPKALEEKIRTTETQVLVASAQKKLLEERLKLVSELWDAGIKAELLYKKNPKLLNQLQYCEEAGIPLVAIIGEQELKDGVIKLRSVTSREEVDVRREDLVEEIKRRTGQPLCIC

SEQ ID NO: 106 - protein, 211 aa, Homo sapiens
MAERAALEELVKLQGERVRGLKQQKASAELIEEEVAKLLKLKAQLGPDESKQKFVLKTPKGTRDYSPRQMAVREKVFDVIIRCFKRHGAEVIDTPVFELKALEEKIRTTETQVLVASAQKKLLEERLKLVSELWDAGIKAELLYKKNPKLLNQLQYCEEAGIPLVAIIGEQELKDGVIKLRSVTSREEVDVRREDLVEEIKRRTGQPLCIC

SEQ ID NO: 107 - protein, 141 aa, Homo sapiens [sequence omitted]

SEQ ID NO: 108 - protein, 143 aa, Homo sapiens
CLKIMCEILSSLQIGDFLVKVNDRRILDGMFAICGVSDSKFRTICSSVDKLDKVSWEEVKNEMVGEKGLAPEVADRIGDYVQQHGGVSLVEQLLQDPKLSQNKQALEGLGDLKLLFEYLTLFGIDDKISFDLSLARGLDYYTG

SEQ ID NO: 109 - protein, 506 aa, Homo sapiens
MPLLGLLPRRAWASLLSQLLRPPCASCTGAVRCQSQVAEAVLTSQLKAHQEKPNFIIKTPKGTRDLSPQHMVVREKILDLVISCFKRHGAKGMDTPAFELKETLTEKYGEDSGLMYDLKDQGGELLSLRYDLTVPFARYLAMNKVKKMKRYHVGKVWRRESPTIVQGRYREFCQCDFDIAGQFDPMIPDAECLKIMCEILSGLQLGDFLIKVNDRRIVDGMFAVCGVPESKFRAICSSIDKLDKMAWKDVRHEMVVKKGLAPEVADRIGDYVQCHGGVSLVEQMFQDPRLSQNKQALEGLGDLKLLFEYLTLFGIADKISFDLSLARGLDYYTGVIYEAVLLQTPTQAGEEPLNVGSVAAGGRYDGLVGMFDPKGHKVPCVGLSIGVERIFYIVEQRMKTKGEKVRTTETQVFVATPQKNFLQERLKLIAELWDSGIKAEMLYKNNPKLLTQLHYCESTGIPLVVIIGEQELKEGVIKIRSVASREEVAIKRENFVAEIQKRLSES

SEQ ID NO: 110 - protein, 509 aa, Mus musculus
MADRAALEELVRLQGAHVRGLKEQKASAEQIEEEVTKLLKLKAQLGQDEGKQKFVLKTPKGTRDYSPRQMAVREKVFDVIIRCFKRHGAEVIDTPVFELKETLTGKYGEDSKLIYDLKDQGGELLSLRYDLTVPFARYLAMNKLTNIKRYHIAKVYRRDNPAMTRGRYREFYQCDFDIAGQFDPMIPDAECLKIMCEILSSLQIGNFLVKVNDRRILDGMFAVCGVPDSKFRTICSSVDKLDKVSWEEVKNEMVGEKGLAPEVADRIGDYVQQHGGVSLVEQLLQDPKLSQNKQAVEGLGDLKLLFEYLILFGIDDKISFDLSLARGLDYYTGVIYEAVLLQMPTQAGEEPLGVGSIAAGGRYDGLVGMFDPKGRKVPCVGLSIGVERIFSIVEQRLEASEEKVRTTETQVLVASAQKKLLEERLKLVSELWDAGIKAELLYKKNPKLLNQLQYWEEAGIPLVAIIGEQELRDGVIKLRSVASREEVDVRREDLVEEIRRRTNQPLSTC

SEQ ID NO: 111 - protein, 509 aa, Canis lupus familiaris
MAERAALEELVRLQGERVRGLKQQKASAEQIEEEVAKLLKLKAQLGPDEGKQKFVLKTPKGTRDYSPRQMAVREKVFDVIISCFKRHGAEVIDTPVFELKETLTGKYGEDSKLIYDLKDQGGELLSLRYDLTVPFARYLAMNKLTNIKRYHIAKVYRRDNPAMTRGRYREFYQCDFDIAGQFDPMIPDAECLEIMCEILRSLQIGDFLVKVNDRRILDGMFAICGVPDSKFRTICSSVDKLDKVSWEEVKNEMVGEKGLAPEVADHIGDYVQQHGGISLVEQLLQDPELSQNKQALEGLGDLKLLFEYLTLFGIADKISFDLSLARGLDYYTGVIYEAVLLQTPVQAGEEPLGVGSVAAGGRYDGLVGMFDPKGRKVPCVGLSIGVERIFSIVEQRLEATEEKVRTTETQVLVASAQKKLLEERLKLVSELWNAGIKAELLYKKNPKLLNQLQYCEEAGIPLVAIIGEQELKDGVIKLRSVASREEVDVPREDLVEEIKRRTSQPFCIC

SEQ ID NO: 112 - protein, 509 aa, Bos taurus
MADRAALEDLVRVQGERVRGLKQQKASAEQIEEEVAKLLKLKAQLGPDEGKPKFVLKTPKGTRDYSPRQMAVREKVFDVIISCFKRHGAEVIDTPVFELKETLTGKYGEDSKLIYDLKDQGGELLSLRYDLTVPFARYLAMNKLTNIKRYHIAKVYRRDNPAMTRGRYREFYQCDFDIAGQFDPMLPDAECLKIMCEILSSLQIGDFLVKVNDRRILDGMFAICGVPDSKFRTICSSVDKLDKVSWEEVKNEMVGEKGLAPEVADRIGDYVQQHGGVSLVEQLLQDPKLSQNKQALEGLGDLKLLFEYLTLFGIADKISFDLSLARGLDYYTGVIYEAVLLQPPARAGEEPLGVGSVAAGGRYDGLVGMFDPKGRKVPCVGLSIGVERIFSIVEQRLEALEEKVRTTETQVLVASAQKKLLEERLKLISELWDAGIKAELLYKKNPKLLNQLQYCEETGIPLVAIIGEQELKDGVIKLRSVASREEVDVRREDLVEEIKRRTSQPLCIC

SEQ ID NO: 113 - protein, 508 aa, Rattus norvegicus
MADRAALEELVRLQGAHVRGLKEQKASAEQIEEEVTKLLKLKAQLGHDEGKQKFVLKTPKGTRDYSPRQMAVREKVFDVIIRCFKRHGAEVIDTPVFELKETLTGKYGEDSKLIYDLKDQGGELLSLRYDLTVPFARYLAMNKLTNIKRYHIAKVYRRDNPAMTRGRYREFYQCDFDIAGQFDPMIPDAECLKIMCEILSSLQIGNFQVKVNDRRILDGMFAVCGVPDSKFRTICSSVDKLDKVSWEEVKNEMVGEKGLAPEVADRIGDYVQQHGGVSLVEQLLQDPKLSQNKQAVEGLGDLKLLFEYLTLFGIDDKISFDLSLARGLDYYTGVIYEAVLLQMPTQAGEEPLGVGSIAAGGRYDGLVGMFDPKGRKVPCVGLSIGVERIFSIVEQKLEASEEKVRTTETQVLVASAQKKLLEERLKLISELWDAGIKAELLYKKNPKLLNQLQYCEEAGIPLVAIIGEQELKDGVIKLRSVTSREEVDVRREDLVEEIRRRTSQPLSM

SEQ ID NO: 114 - protein, 500 aa, Gallus gallus
MADEAAVRQQAEVVRRLKQDKAEPDEIAKEVAKLLEMKAHLGGDEGKHKFVLKTPKGTRDYGPKQMAIRERVFSAIIACFKRHGAEVIDTPVFELKETLTGKYGEDSKLIYDLKDQGGELLSLRYDLTVPFARYLAMNKITNIKRYHIAKVYRRDNPAMTRGRYREFYQCDFDIAGQFDPMIPDAECLKIVQEILSDLQLGDFLIKVNDRRILDGMFAVCGVPDSKFRTICSSVDKLDKMPWEEVRNEMVGEKGLSPEAADRIGEYVQLHGGMDLIEQLLQDPKLSQNKLVKEGLGDMKLLFEYLTLFGITGKISFDLSLARGLDYYTGVIYEAVLLQQNDHGEESVSVGSVAGGGRYDGLVGMFDPKGRKVPCVGISIGIERIFSILEQRVEASEEKIRTTETQVLVASAQKKLLEERLKLISELWDAGIKAEVLYKKNPKLLNQLQYCEDTGIPLVAIVGEQELKDGVVKLRVVATGEEVNIRRESLVEEIRRRTNQL

SEQ ID NO: 115 - protein, 437 aa, Danio rerio
MAALGLVSMRLCAGLMGRRSAVRLHSLRVCSGMTISQIDEEVARLLQLKAQLGGDEGKHVFVLKTAKGTRDYNPKQMAIREKVFNIIINCFKRHGAETIDSPVFELKETLTGKYGEDSKLIYDLKDQGGELLSLRYDLTVPFARYLAMNKITNIKRYHIAKVYRRDNPAMTRGRYREFYQCDFDIAGQYDAMIPDAECLKLVYEILSELDLGDFRIKVNDRRILDGMFAICGVPDEKFRTICSTVDKLDKLAWEEVKKEMVNEKGLSEEVADRIRDYVSMQGGKDLAERLLQDPKLSQSKQACAGITDMKLLFSYLELFQITDKVVFDLSLARGLDYYTGVIYEAILTQANPAPASTPAEQNGAEDAGVSVGSVAGGGRYDGLVGMFDPKAGKCPVWGSALALRGSSPSWSRRQSCLQRRCAPLKLKCLWLQHRRTF

SEQ ID NO: 116 - protein, 435 aa, Macaca fascicularis
MAERAALEELVKLQGERVRGLKQQQASAELIEEEVGKLLKLKAQLGPDESKQKFVLKTPKGTRDYSPRQMAVREKVFDVIIRCFKRHGAEVIDTPVFELKDFDIAGNFDPMIPDAECLKIMCEILSSLQIGDFLVKVNDRRILDGMFAICGVSDSKFRTICSSVDKLDKVSWEEVKNEMVGEKGLAPEVADRIGDYVQQHGGVSLVEQLLQDPKLSQNKQALEGLGDLKLLFEYLTLFGIDDKISFDLSLARGLDYYTGVIYEAVLLQTPAQAGEEPLGVGSVAAGGRYDGLVGMFDPKGRKVPCVGLSIGVERIFSIVEQRLEALEEKVRTTETQVLVASAQKKLLEERLKLVSELWDAGIKAELLYKKNPKLLNQLQYCEEAGIPLVAIIGEQELKDGVIKLRSVTSREEVNVRREDLVEEIKRRTGQLLRIC

SEQ ID NO: 117 - protein, 138 aa, Artificial Sequence
  Consensus HRS WHEP sequence
  MOD_RES (1)..(50): Xaa is any amino acid or absent
  misc_feature (52)..(56): Xaa can be any naturally occurring amino acid
  MOD_RES (57)..(58): Xaa is any amino acid or absent
  MOD_RES (61)..(62): Xaa is any amino acid
  MOD_RES (65)..(65): Xaa is any amino acid
  MOD_RES (68)..(69): Xaa is any amino acid
  misc_feature (72)..(78): Xaa can be any naturally occurring amino acid
  MOD_RES (79)..(80): Xaa is any amino acid or absent
  MOD_RES (82)..(83): Xaa is any amino acid
  MOD_RES (86)..(86): Xaa is any amino acid
  MOD_RES (89)..(138): Xaa is any amino acid or absent
XXXXXXXXXXXXXXXXXXXXXXXXXXXXXXXXXXXXXXXXXXXXXXXXXXLXXXXXXXQGXXVRXLKXXKAXXXXXXXXXVXXLLXLKXXXXXXXXXXXXXXXXXXXXXXXXXXXXXXXXXXXXXXXXXXXXXXXXXX

SEQ ID NO: 118 - protein, 61 aa, Artificial Sequence
  Made in Lab:  cysteine modified HRS polypeptide
MCAERAALEELVKLQGERVRGLKQQKASAELIEEEVAKLLKLKAQLGPDESKQKFVLKTPK

SEQ ID NO: 119 - protein, 60 aa, Artificial Sequence
  Made in Lab:  cysteine modified HRS polypeptide
MAERAALEELVKLQGERVRGLKQQKCSAELIEEEVAKLLKLKAQLGPDESKQKFVLKTPK

SEQ ID NO: 120 - protein, 61 aa, Artificial Sequence
  Made in Lab:  cysteine modified HRS polypeptide
MAERAALEELVKLQGERVRGLKQQKASAELIEEEVAKLLKLKAQLGPDESKQKFVLKTPKC

SEQ ID NO: 121 - protein, 506 aa, Artificial Sequence
  Made in Lab: modified HRS polypeptide to remove surface exposed cysteines
MAERAALEELVKLQGERVRGLKQQKASAELIEEEVAKLLKLKAQLGPDESKQKFVLKTPKGTRDYSPRQMAVREKVFDVIIRCFKRHGAEVIDTPVFELKETLMGKYGEDSKLIYDLKDQGGELLSLRYDLTVPFARYLAMNKLTNIKRYHIAKVYRRDNPAMTRGRYREFYQADFDIAGNFDPMIPDAECLKIMCEILSSLQIGDFLVKVNDRRILDGMFAICGVSDSKFRTICSSVDKLDKVSWEEVKNEMVGEKGLAPEVADRIGDYVQQHGGVSLVEQLLQDPKLSQNKQALEGLGDLKLLFEYLTLFGIDDKISFDLSLARGLDYYTGVIYEAVLLQTPAQAGEEPLGVGSVAAGGRYDGLVGMFDPKGRKVPCVGLSIGVERIFSIVEQRLEALEEKIRTTETQVLVASAQKKLLEERLKLVSELWDAGIKAELLYKKNPKLLNQLQYCEEAGIPLVAIIGEQELKDGVIKLRSVTSREEVDVRREDLVEEIKRRTGQPL

SEQ ID NO: 122 - protein, 506 aa, Artificial Sequence
  Made in Lab: modified HRS polypeptide to remove surface exposed cysteines
MAERAALEELVKLQGERVRGLKQQKASAELIEEEVAKLLKLKAQLGPDESKQKFVLKTPKGTRDYSPRQMAVREKVFDVIIRCFKRHGAEVIDTPVFELKETLMGKYGEDSKLIYDLKDQGGELLSLRYDLTVPFARYLAMNKLTNIKRYHIAKVYRRDNPAMTRGRYREFYQVDFDIAGNFDPMIPDAECLKIMCEILSSLQIGDFLVKVNDRRILDGMFAICGVSDSKFRTICSSVDKLDKVSWEEVKNEMVGEKGLAPEVADRIGDYVQQHGGVSLVEQLLQDPKLSQNKQALEGLGDLKLLFEYLTLFGIDDKISFDLSLARGLDYYTGVIYEAVLLQTPAQAGEEPLGVGSVAAGGRYDGLVGMFDPKGRKVPCVGLSIGVERIFSIVEQRLEALEEKIRTTETQVLVASAQKKLLEERLKLVSELWDAGIKAELLYKKNPKLLNQLQYCEEAGIPLVAIIGEQELKDGVIKLRSVTSREEVDVRREDLVEEIKRRTGQPL

SEQ ID NO: 123 - protein, 506 aa, Artificial Sequence
  Made in Lab: modified HRS polypeptide to remove surface exposed cysteines
MAERAALEELVKLQGERVRGLKQQKASAELIEEEVAKLLKLKAQLGPDESKQKFVLKTPKGTRDYSPRQMAVREKVFDVIIRCFKRHGAEVIDTPVFELKETLMGKYGEDSKLIYDLKDQGGELLSLRYDLTVPFARYLAMNKLTNIKRYHIAKVYRRDNPAMTRGRYREFYQCDFDIAGNFDPMIPDAEALKIMCEILSSLQIGDFLVKVNDRRILDGMFAICGVSDSKFRTICSSVDKLDKVSWEEVKNEMVGEKGLAPEVADRIGDYVQQHGGVSLVEQLLQDPKLSQNKQALEGLGDLKLLFEYLTLFGIDDKISFDLSLARGLDYYTGVIYEAVLLQTPAQAGEEPLGVGSVAAGGRYDGLVGMFDPKGRKVPCVGLSIGVERIFSIVEQRLEALEEKIRTTETQVLVASAQKKLLEERLKLVSELWDAGIKAELLYKKNPKLLNQLQYCEEAGIPLVAIIGEQELKDGVIKLRSVTSREEVDVRREDLVEEIKRRTGQPL

SEQ ID NO: 124 - protein, 506 aa, Artificial Sequence
  Made in Lab: modified HRS polypeptide to remove surface exposed cysteines
MAERAALEELVKLQGERVRGLKQQKASAELIEEEVAKLLKLKAQLGPDESKQKFVLKTPKGTRDYSPRQMAVREKVFDVIIRCFKRHGAEVIDTPVFELKETLMGKYGEDSKLIYDLKDQGGELLSLRYDLTVPFARYLAMNKLTNIKRYHIAKVYRRDNPAMTRGRYREFYQCDFDIAGNFDPMIPDAESLKIMCEILSSLQIGDFLVKVNDRRILDGMFAICGVSDSKFRTICSSVDKLDKVSWEEVKNEMVGEKGLAPEVADRIGDYVQQHGGVSLVEQLLQDPKLSQNKQALEGLGDLKLLFEYLTLFGIDDKISFDLSLARGLDYYTGVIYEAVLLQTPAQAGEEPLGVGSVAAGGRYDGLVGMFDPKGRKVPCVGLSIGVERIFSIVEQRLEALEEKIRTTETQVLVASAQKKLLEERLKLVSELWDAGIKAELLYKKNPKLLNQLQYCEEAGIPLVAIIGEQELKDGVIKLRSVTSREEVDVRREDLVEEIKRRTGQPL

SEQ ID NO: 125 - protein, 506 aa, Artificial Sequence
  Made in Lab: modified HRS polypeptide to remove surface exposed cysteines
MAERAALEELVKLQGERVRGLKQQKASAELIEEEVAKLLKLKAQLGPDESKQKFVLKTPKGTRDYSPRQMAVREKVFDVIIRCFKRHGAEVIDTPVFELKETLMGKYGEDSKLIYDLKDQGGELLSLRYDLTVPFARYLAMNKLTNIKRYHIAKVYRRDNPAMTRGRYREFYQCDFDIAGNFDPMIPDAEVLKIMCEILSSLQIGDFLVKVNDRRILDGMFAICGVSDSKFRTICSSVDKLDKVSWEEVKNEMVGEKGLAPEVADRIGDYVQQHGGVSLVEQLLQDPKLSQNKQALEGLGDLKLLFEYLTLFGIDDKISFDLSLARGLDYYTGVIYEAVLLQTPAQAGEEPLGVGSVAAGGRYDGLVGMFDPKGRKVPCVGLSIGVERIFSIVEQRLEALEEKIRTTETQVLVASAQKKLLEERLKLVSELWDAGIKAELLYKKNPKLLNQLQYCEEAGIPLVAIIGEQELKDGVIKLRSVTSREEVDVRREDLVEEIKRRTGQPL

SEQ ID NO: 126 - protein, 506 aa, Artificial Sequence
  Made in Lab: modified HRS polypeptide to remove surface exposed cysteines
MAERAALEELVKLQGERVRGLKQQKASAELIEEEVAKLLKLKAQLGPDESKQKFVLKTPKGTRDYSPRQMAVREKVFDVIIRCFKRHGAEVIDTPVFELKETLMGKYGEDSKLIYDLKDQGGELLSLRYDLTVPFARYLAMNKLTNIKRYHIAKVYRRDNPAMTRGRYREFYQCDFDIAGNFDPMIPDAECLKIMCEILSSLQIGDFLVKVNDRRILDGMFAISGVSDSKFRTICSSVDKLDKVSWEEVKNEMVGEKGLAPEVADRIGDYVQQHGGVSLVEQLLQDPKLSQNKQALEGLGDLKLLFEYLTLFGIDDKISFDLSLARGLDYYTGVIYEAVLLQTPAQAGEEPLGVGSVAAGGRYDGLVGMFDPKGRKVPCVGLSIGVERIFSIVEQRLEALEEKIRTTETQVLVASAQKKLLEERLKLVSELWDAGIKAELLYKKNPKLLNQLQYCEEAGIPLVAIIGEQELKDGVIKLRSVTSREEVDVRREDLVEEIKRRTGQPL

SEQ ID NO: 127 - protein, 506 aa, Artificial Sequence
  Made in Lab: modified HRS polypeptide to remove surface exposed cysteines
MAERAALEELVKLQGERVRGLKQQKASAELIEEEVAKLLKLKAQLGPDESKQKFVLKTPKGTRDYSPRQMAVREKVFDVIIRCFKRHGAEVIDTPVFELKETLMGKYGEDSKLIYDLKDQGGELLSLRYDLTVPFARYLAMNKLTNIKRYHIAKVYRRDNPAMTRGRYREFYQCDFDIAGNFDPMIPDAECLKIMCEILSSLQIGDFLVKVNDRRILDGMFAICGVSDSKFRTISSSVDKLDKVSWEEVKNEMVGEKGLAPEVADRIGDYVQQHGGVSLVEQLLQDPKLSQNKQALEGLGDLKLLFEYLTLFGIDDKISFDLSLARGLDYYTGVIYEAVLLQTPAQAGEEPLGVGSVAAGGRYDGLVGMFDPKGRKVPCVGLSIGVERIFSIVEQRLEALEEKIRTTETQVLVASAQKKLLEERLKLVSELWDAGIKAELLYKKNPKLLNQLQYCEEAGIPLVAIIGEQELKDGVIKLRSVTSREEVDVRREDLVEEIKRRTGQPL

SEQ ID NO: 128 - protein, 19 aa, Homo sapiens
VPSTPPTPSPSTPPTPSPS

SEQ ID NO: 129 - protein, 101 aa, Homo sapiens
CCHPRLSLHRPALEDLLLGSEANLTCTLTGLRDASGVTFTWTPSSGKSAVQGPPERDLCGCYSVSSVLPGCAEPWNHGKTFTCTAAYPESKTPLTATLSKS

SEQ ID NO: 130 - protein, 131 aa, Homo sapiens
GNTFRPEVHLLPPPSEELALNELVTLTCLARGFSPKDVLVRWLQGSQELPREKYLTWASRQEPSQGTTTFAVTSILRVAAEDWKKGDTFSCMVGHEALPLAFTQKTIDRLAGKPTHVNVSVVMAEVDGTCY

SEQ ID NO: 131 - protein, 6 aa, Homo sapiens
VPPPPP

SEQ ID NO: 132 - protein, 101 aa, Homo sapiens
CCHPRLSLHRPALEDLLLGSEANLTCTLTGLRDASGATFTWTPSSGKSAVQGPPERDLCGCYSVSSVLPGCAQPWNHGETFTCTAAHPELKTPLTANITKS

SEQ ID NO: 133 - protein, 131 aa, Homo sapiens; identical to SEQ ID NO: 130

SEQ ID NO: 134 - protein, 58 aa, Homo sapiens
ESPKAQASSVPTAQPQAEGSLAKATTAPATTRNTGRGGEEKKKEKEKEEQEERETKTP

SEQ ID NO: 135 - protein, 108 aa, Homo sapiens
ECPSHTQPLGVYLLTPAVQDLWLRDKATFTCFVVGSDLKDAHLTWEVAGKVPTGGVEEGLLERHSNGSQSQHSRLTLPRSLWNAGTSVTCTLNHPSLPPQRLMALREP

SEQ ID NO: 136 - protein, 117 aa, Homo sapiens
AAQAPVKLSLNLLASSDPPEAASWLLCEVSGFSPPNILLMWLEDQREVNTSGFAPARPPPQPRSTTFWAWSVLRVPAPPSPQPATYTCVVSHEDSRTLLNASRSLEVSYVTDHGPMK

SEQ ID NO: 137 - protein, 107 aa, Homo sapiens
VCSRDFTPPTVKILQSSCDGGGHFPPTIQLLCLVSGYTPGTINITWLEDGQVMDVDLSTASTTQEGELASTQSELTLSQKHWLSDRTYTCQVTYQGHTFEDSTKKCA

SEQ ID NO: 138 - protein, 108 aa, Homo sapiens
DSNPRGVSAYLSRPSPFDLFIRKSPTITCLVVDLAPSKGTVNLTWSRASGKPVNHSTRKEEKQRNGTLTVTSTLPVGTRDWIEGETYQCRVTHPHLPRALMRSTTKTS

SEQ ID NO: 139 - protein, 110 aa, Homo sapiens
GPRAAPEVYAFATPEWPGSRDKRTLACLIQNFMPEDISVQWLHNEVQLPDARHSTTQPRKTKGSGFFVFSRLEVTRAEWEQKDEFICRAVHEAASPSQTVQRAVSVNPGK

SEQ ID NO: 140 - protein, 15 aa, Homo sapiens
EPKSCDKTHTCPPCP

SEQ ID NO: 141 - protein, 11 aa, Homo sapiens
SDKTHTCPPCP

SEQ ID NO: 142 - protein, 110 aa, Homo sapiens
APELLGGPSVFLFPPKPKDTLMISRTPEVTCVVVDVSHEDPEVKFNWYVDGVEVHNAKTKPREEQYNSTYRVVSVLTVLHQDWLNGKEYKCKVSNKALPAPIEKTISKAK

SEQ ID NO: 143 - protein, 107 aa, Homo sapiens
GQPREPQVYTLPPSRDELTKNQVSLTCLVKGFYPSDIAVEWESNGQPENNYKTTPPVLDSDGSFFLYSKLTVDKSRWQQGNVFSCSVMHEALHNHYTQKSLSLSPGK

SEQ ID NO: 144 - protein, 229 aa, Homo sapiens
MSDKTHTCPPCPAPELLGGPSVFLFPPKPKDTLMISRTPEVTCVVVDVSHEDPEVKFNWYVDGVEVHNAKTKPREEQYNSTYRVVSVLTVLHQDWLNGKEYKCKVSNKALPAPIEKTISKAKGQPREPQVYTLPPSREEMTKNQVSLTCLVKGFYPSDIAVEWESNGQPENNYKTTPPVLDSDGSFFLYSKLTVDKSRWQQGNVFSCSVMHEALHNHYTQKSLSLSPGK

SEQ ID NO: 145 - protein, 12 aa, Homo sapiens
ERKCCVECPPCP

SEQ ID NO: 146 - protein, 109 aa, Homo sapiens
APPVAGPSVFLFPPKPKDTLMISRTPEVTCVVVDVSHEDPEVQFNWYVDGVEVHNAKTKPREEQFNSTFRVVSVLTVVHQDWLNGKEYKCKVSNKGLPAPIEKTISKTK

SEQ ID NO: 147 - protein, 107 aa, Homo sapiens
GQPREPQVYTLPPSREEMTKNQVSLTCLVKGFYPSDIAVEWESNGQPENNYKTTPPMLDSDGSFFLYSKLTVDKSRWQQGNVFSCSVMHEALHNHYTQKSLSLSPGK

SEQ ID NO: 148 - protein, 62 aa, Homo sapiens
ELKTPLGDTTHTCPRCPEPKSCDTPPPCPRCPEPKSCDTPPPCPRCPEPKSCDTPPPCPRCP

SEQ ID NO: 149 - protein, 110 aa, Homo sapiens
APELLGGPSVFLFPPKPKDTLMISRTPEVTCVVVDVSHEDPEVQFKWYVDGVEVHNAKTKPREEQYNSTFRVVSVLTVLHQDWLNGKEYKCKVSNKALPAPIEKTISKTK

SEQ ID NO: 150 - protein, 107 aa, Homo sapiens
GQPREPQVYTLPPSREEMTKNQVSLTCLVKGFYPSDIAVEWESSGQPENNYNTTPPMLDSDGSFFLYSKLTVDKSRWQQGNIFSCSVMHEALHNRFTQKSLSLSPGK

SEQ ID NO: 151 - protein, 12 aa, Homo sapiens
ESKYGPPCPSCP

SEQ ID NO: 152 - protein, 110 aa, Homo sapiens
APEFLGGPSVFLFPPKPKDTLMISRTPEVTCVVVDVSQEDPEVQFNWYVDGVEVHNAKTKPREEQFNSTYRVVSVLTVLHQDWLNGKEYKCKVSNKGLPSSIEKTISKAK

SEQ ID NO: 153 - protein, 107 aa, Homo sapiens
GQPREPQVYTLPPSQEEMTKNQVSLTCLVKGFYPSDIAVEWESNGQPENNYKTTPPVLDSDGSFFLYSRLTVDKSRWQEGNVFSCSVMHEALHNHYTQKSLSLSLGK

SEQ ID NO: 154 - protein, 112 aa, Homo sapiens
VIAELPPKVSVFVPPRDGFFGNPRKSKLICQATGFSPRQIQVSWLREGKQVGSGVTTDQVQAEAKESGPTTYKVTSTLTIKESDWLGQSMFTCRVDHRGLTFQQNASSMCVP

SEQ ID NO: 155 - protein, 106 aa, Homo sapiens
DQDTAIRVFAIPPSFASIFLTKSTKLTCLVTDLTTYDSVTISWTRQNGEAVKTHTNISESHPNATFSAVGEASICEDDWNSGERFTCTVTHTDLPSPLKQTISRPK

SEQ ID NO: 156 - protein, 131 aa, Homo sapiens
GVALHRPDVYLLPPAREQLNLRESATITCLVTGFSPADVFVQWMQRGQPLSPEKYVTSAPMPEPQAPGRYFAHSILTVSEEEWNTGETYTCVVAHEALPNRVTERTVDKSTGKPTLYNVSLVMSDTAGTCY

SEQ ID NO: 157 - protein, 287 aa, Artificial Sequence
  Made in Lab: HRS-Fc fusion protein
MDKTHTCPPCPAPELLGGPSVFLFPPKPKDTLMISRTPEVTCVVVDVSHEDPEVKFNWYVDGVEVHNAKTKPREEQYNSTYRVVSVLTVLHQDWLNGKEYKCKVSNKALPAPIEKTISKAKGQPREPQVYTLPPSRDELTKNQVSLTCLVKGFYPSDIAVEWESNGQPENNYKTTPPVLDSDGSFFLYSKLTVDKSRWQQGNVFSCSVMHEALHNHYTQKSLSLSPGKAERAALEELVKLQGERVRGLKQQKASAELIEEEVAKLLKLKAQLGPDESKQKFVLKTPK

SEQ ID NO: 158 - protein, 288 aa, Artificial Sequence
  Made in Lab: HRS-Fc fusion protein
MSDKTHTCPPCPAPELLGGPSVFLFPPKPKDTLMISRTPEVTCVVVDVSHEDPEVKFNWYVDGVEVHNAKTKPREEQYNSTYRVVSVLTVLHQDWLNGKEYKCKVSNKALPAPIEKTISKAKGQPREPQVYTLPPSREEMTKNQVSLTCLVKGFYPSDIAVEWESNGQPENNYKTTPPVLDSDGSFFLYSKLTVDKSRWQQGNVFSCSVMHEALHNHYTQKSLSLSPGKAERAALEELVKLQGERVRGLKQQKASAELIEEEVAKLLKLKAQLGPDESKQKFVLKTPK

SEQ ID NO: 159 - protein, 288 aa, Artificial Sequence
  Made in Lab: HRS-Fc fusion protein
MAERAALEELVKLQGERVRGLKQQKASAELIEEEVAKLLKLKAQLGPDESKQKFVLKTPKSDKTHTCPPCPAPELLGGPSVFLFPPKPKDTLMISRTPEVTCVVVDVSHEDPEVKFNWYVDGVEVHNAKTKPREEQYNSTYRVVSVLTVLHQDWLNGKEYKCKVSNKALPAPIEKTISKAKGQPREPQVYTLPPSREEMTKNQVSLTCLVKGFYPSDIAVEWESNGQPENNYKTTPPVLDSDGSFFLYSKLTVDKSRWQQGNVFSCSVMHEALHNHYTQKSLSLSPGK

SEQ ID NO: 160 - protein, 288 aa, Artificial Sequence; identical to SEQ ID NO: 158
  Made in Lab: HRS-Fc fusion protein

SEQ ID NO: 161 - protein, 288 aa, Artificial Sequence; identical to SEQ ID NO: 159
  Made in Lab: HRS-Fc fusion protein

SEQ ID NO: 162 - protein, 268 aa, Artificial Sequence
  Made in Lab: HRS-Fc fusion protein
MSDKTHTCPPCPAPELLGGPSVFLFPPKPKDTLMISRTPEVTCVVVDVSHEDPEVKFNWYVDGVEVHNAKTKPREEQYNSTYRVVSVLTVLHQDWLNGKEYKCKVSNKALPAPIEKTISKAKGQPREPQVYTLPPSREEMTKNQVSLTCLVKGFYPSDIAVEWESNGQPENNYKTTPPVLDSDGSFFLYSKLTVDKSRWQQGNVFSCSVMHEALHNHYTQKSLSLSPGKAERAALEELVKLQGERVRGLKQQKASAELIEEEVAKLLK

SEQ ID NO: 163 - protein, 273 aa, Artificial Sequence
  Made in Lab: HRS-Fc fusion protein
MSDKTHTCPPCPAPELLGGPSVFLFPPKPKDTLMISRTPEVTCVVVDVSHEDPEVKFNWYVDGVEVHNAKTKPREEQYNSTYRVVSVLTVLHQDWLNGKEYKCKVSNKALPAPIEKTISKAKGQPREPQVYTLPPSREEMTKNQVSLTCLVKGFYPSDIAVEWESNGQPENNYKTTPPVLDSDGSFFLYSKLTVDKSRWQQGNVFSCSVMHEALHNHYTQKSLSLSPGKAERAALEELVKLQGERVRGLKQQKASAELIEEEVAKLLKLKAQL

SEQ ID NO: 164 - protein, 278 aa, Artificial Sequence
  Made in Lab: HRS-Fc fusion protein
MSDKTHTCPPCPAPELLGGPSVFLFPPKPKDTLMISRTPEVTCVVVDVSHEDPEVKFNWYVDGVEVHNAKTKPREEQYNSTYRVVSVLTVLHQDWLNGKEYKCKVSNKALPAPIEKTISKAKGQPREPQVYTLPPSREEMTKNQVSLTCLVKGFYPSDIAVEWESNGQPENNYKTTPPVLDSDGSFFLYSKLTVDKSRWQQGNVFSCSVMHEALHNHYTQKSLSLSPGKAERAALEELVKLQGERVRGLKQQKASAELIEEEVAKLLKLKAQLGPDES

SEQ ID NO: 165 - protein, 283 aa, Artificial Sequence
  Made in Lab: HRS-Fc fusion protein
MSDKTHTCPPCPAPELLGGPSVFLFPPKPKDTLMISRTPEVTCVVVDVSHEDPEVKFNWYVDGVEVHNAKTKPREEQYNSTYRVVSVLTVLHQDWLNGKEYKCKVSNKALPAPIEKTISKAKGQPREPQVYTLPPSREEMTKNQVSLTCLVKGFYPSDIAVEWESNGQPENNYKTTPPVLDSDGSFFLYSKLTVDKSRWQQGNVFSCSVMHEALHNHYTQKSLSLSPGKAERAALEELVKLQGERVRGLKQQKASAELIEEEVAKLLKLKAQLGPDESKQKFV

SEQ ID NO: 166 - protein, 294 aa, Artificial Sequence
  Made in Lab: HRS-Fc fusion protein
MSDKTHTCPPCPAPELLGGPSVFLFPPKPKDTLMISRTPEVTCVVVDVSHEDPEVKFNWYVDGVEVHNAKTKPREEQYNSTYRVVSVLTVLHQDWLNGKEYKCKVSNKALPAPIEKTISKAKGQPREPQVYTLPPSREEMTKNQVSLTCLVKGFYPSDIAVEWESNGQPENNYKTTPPVLDSDGSFFLYSKLTVDKSRWQQGNVFSCSVMHEALHNHYTQKSLSLSPGKAERAALEELVKLQGERVRGLKQQKASAELIEEEVAKLLKLKAQLGPDESKQKFVLKTPKGTRDYS

SEQ ID NO: 167 - protein, 268 aa, Artificial Sequence
  Made in Lab: HRS-Fc fusion protein
MAERAALEELVKLQGERVRGLKQQKASAELIEEEVAKLLKSDKTHTCPPCPAPELLGGPSVFLFPPKPKDTLMISRTPEVTCVVVDVSHEDPEVKFNWYVDGVEVHNAKTKPREEQYNSTYRVVSVLTVLHQDWLNGKEYKCKVSNKALPAPIEKTISKAKGQPREPQVYTLPPSREEMTKNQVSLTCLVKGFYPSDIAVEWESNGQPENNYKTTPPVLDSDGSFFLYSKLTVDKSRWQQGNVFSCSVMHEALHNHYTQKSLSLSPGK

SEQ ID NO: 168 - protein, 273 aa, Artificial Sequence
  Made in Lab: HRS-Fc fusion protein
MAERAALEELVKLQGERVRGLKQQKASAELIEEEVAKLLKLKAQLSDKTHTCPPCPAPELLGGPSVFLFPPKPKDTLMISRTPEVTCVVVDVSHEDPEVKFNWYVDGVEVHNAKTKPREEQYNSTYRVVSVLTVLHQDWLNGKEYKCKVSNKALPAPIEKTISKAKGQPREPQVYTLPPSREEMTKNQVSLTCLVKGFYPSDIAVEWESNGQPENNYKTTPPVLDSDGSFFLYSKLTVDKSRWQQGNVFSCSVMHEALHNHYTQKSLSLSPGK

SEQ ID NO: 169 - protein, 278 aa, Artificial Sequence
  Made in Lab: HRS-Fc fusion protein
MAERAALEELVKLQGERVRGLKQQKASAELIEEEVAKLLKLKAQLGPDESSDKTHTCPPCPAPELLGGPSVFLFPPKPKDTLMISRTPEVTCVVVDVSHEDPEVKFNWYVDGVEVHNAKTKPREEQYNSTYRVVSVLTVLHQDWLNGKEYKCKVSNKALPAPIEKTISKAKGQPREPQVYTLPPSREEMTKNQVSLTCLVKGFYPSDIAVEWESNGQPENNYKTTPPVLDSDGSFFLYSKLTVDKSRWQQGNVFSCSVMHEALHNHYTQKSLSLSPGK

SEQ ID NO: 170 - protein, 283 aa, Artificial Sequence
  Made in Lab: HRS-Fc fusion protein
MAERAALEELVKLQGERVRGLKQQKASAELIEEEVAKLLKLKAQLGPDESKQKFVSDKTHTCPPCPAPELLGGPSVFLFPPKPKDTLMISRTPEVTCVVVDVSHEDPEVKFNWYVDGVEVHNAKTKPREEQYNSTYRVVSVLTVLHQDWLNGKEYKCKVSNKALPAPIEKTISKAKGQPREPQVYTLPPSREEMTKNQVSLTCLVKGFYPSDIAVEWESNGQPENNYKTTPPVLDSDGSFFLYSKLTVDKSRWQQGNVFSCSVMHEALHNHYTQKSLSLSPGK

SEQ ID NO: 171 - protein, 294 aa, Artificial Sequence
  Made in Lab: HRS-Fc fusion protein
MAERAALEELVKLQGERVRGLKQQKASAELIEEEVAKLLKLKAQLGPDESKQKFVLKTPKGTRDYSSDKTHTCPPCPAPELLGGPSVFLFPPKPKDTLMISRTPEVTCVVVDVSHEDPEVKFNWYVDGVEVHNAKTKPREEQYNSTYRVVSVLTVLHQDWLNGKEYKCKVSNKALPAPIEKTISKAKGQPREPQVYTLPPSREEMTKNQVSLTCLVKGFYPSDIAVEWESNGQPENNYKTTPPVLDSDGSFFLYSKLTVDKSRWQQGNVFSCSVMHEALHNHYTQKSLSLSPGK

SEQ ID NO: 172 - protein, 347 aa, Artificial Sequence
  Made in Lab: HRS-Fc fusion protein
MSDKTHTCPPCPAPELLGGPSVFLFPPKPKDTLMISRTPEVTCVVVDVSHEDPEVKFNWYVDGVEVHNAKTKPREEQYNSTYRVVSVLTVLHQDWLNGKEYKCKVSNKALPAPIEKTISKAKGQPREPQVYTLPPSREEMTKNQVSLTCLVKGFYPSDIAVEWESNGQPENNYKTTPPVLDSDGSFFLYSKLTVDKSRWQQGNVFSCSVMHEALHNHYTQKSLSLSPGKAERAALEELVKLQGERVRGLKQQKASAELIEEEVAKLLKLKAQLGPDESKQKFVLKTPKAERAALEELVKLQGERVRGLKQQKASAELIEEEVAKLLKLKAQLGPDESKQKFVLKTPK

SEQ ID NO: 173 - protein, 4 aa, Artificial Sequence
  Made in Lab: peptide linker sequence
GSGS

SEQ ID NO: 174 - protein, 4 aa, Artificial Sequence
  Made in Lab: peptide linker sequence
GGSG

SEQ ID NO: 175 - protein, 4 aa, Artificial Sequence
  Made in Lab: peptide linker sequence
GGGS

SEQ ID NO: 176 - protein, 5 aa, Artificial Sequence
  Made in Lab: peptide linker sequence
GGGGS

SEQ ID NO: 177 - protein, 4 aa, Artificial Sequence
  Made in Lab: peptide linker sequence
GNGN

SEQ ID NO: 178 - protein, 4 aa, Artificial Sequence
  Made in Lab: peptide linker sequence
GGNG

SEQ ID NO: 179 - protein, 4 aa, Artificial Sequence
  Made in Lab: peptide linker sequence
GGGN

SEQ ID NO: 180 - protein, 5 aa, Artificial Sequence
  Made in Lab: peptide linker sequence
GGGGN

SEQ ID NO: 181 - protein, 15 aa, Artificial Sequence
  Made in Lab: peptide linker sequence
GGGGSGGGGSGGGGS

SEQ ID NO: 182 - protein, 22 aa, Artificial Sequence
  Made in Lab: peptide linker sequence
GSGGGGSGGGGSGGGGSGGGGS

SEQ ID NO: 183 - protein, 30 aa, Artificial Sequence
  Made in Lab: peptide linker sequence
GGGGSGGGGSGGGGSGGGGSGGGGSGGGGS

SEQ ID NO: 184 - protein, 25 aa, Artificial Sequence
  Made in Lab: peptide linker sequence
DAAAKEAAAKDAAAREAAARDAAAK

SEQ ID NO: 185 - protein, 14 aa, Artificial Sequence
  Made in Lab: peptide linker sequence
NVDHKPSNTKVDKR

SEQ ID NO: 186 - protein, 5 aa, Artificial Sequence
  Made in Lab: peptide linker sequence
DGGGS

SEQ ID NO: 187 - protein, 5 aa, Artificial Sequence
  Made in Lab: peptide linker sequence
TGEKP

SEQ ID NO: 188 - protein, 4 aa, Artificial Sequence
  Made in Lab: peptide linker sequence
GGRR

SEQ ID NO: 189 - protein, 14 aa, Artificial Sequence
  Made in Lab: peptide linker sequence
EGKSSGSGSESKVD

SEQ ID NO: 190 - protein, 18 aa, Artificial Sequence
  Made in Lab: peptide linker sequence
KESGSVSSEQLAQFRSLD

SEQ ID NO: 191 - protein, 8 aa, Artificial Sequence
  Made in Lab: peptide linker sequence
GGRRGGGS

SEQ ID NO: 192 - protein, 9 aa, Artificial Sequence
  Made in Lab: peptide linker sequence
LRQRDGERP

SEQ ID NO: 193 - protein, 12 aa, Artificial Sequence
  Made in Lab: peptide linker sequence
LRQKDGGGSERP

SEQ ID NO: 194 - protein, 16 aa, Artificial Sequence
  Made in Lab: peptide linker sequence
LRQKDGGGSGGGSERP

SEQ ID NO: 195 - protein, 19 aa, Unknown
  Naturally occurring 2A or 2A-like self cleaving peptide
LLNFDLLKLAGDVESNPGP

SEQ ID NO: 196 - protein, 19 aa, Unknown
  Naturally occurring 2A or 2A-like self cleaving peptide
TLNFDLLKLAGDVESNPGP

SEQ ID NO: 197 - protein, 14 aa, Unknown
  Naturally occurring 2A or 2A-like self cleaving peptide
LLKLAGDVESNPGP

SEQ ID NO: 198 - protein, 17 aa, Unknown
  Naturally occurring 2A or 2A-like self cleaving peptide
NFDLLKLAGDVESNPGP

SEQ ID NO: 199 - protein, 20 aa, Unknown
  Naturally occurring 2A or 2A-like self cleaving peptide
QLLNFDLLKLAGDVESNPGP

SEQ ID NO: 200 - protein, 24 aa, Unknown
  Naturally occurring 2A or 2A-like self cleaving peptide
APVKQTLNFDLLKLAGDVESNPGP

SEQ ID NO: 201 - protein, 40 aa, Unknown
  Naturally occurring 2A or 2A-like self cleaving peptide
VTELLYRMKRAETYCPRPLLAIHPTEARHKQKIVAPVKQT

SEQ ID NO: 202 - protein, 18 aa, Unknown
  Naturally occurring 2A or 2A-like self cleaving peptide
LNFDLLKLAGDVESNPGP

SEQ ID NO: 203 - protein, 40 aa, Unknown
  Naturally occurring 2A or 2A-like self cleaving peptide
LLAIHPTEARHKQKIVAPVKQTLNFDLLKLAGDVESNPGP

SEQ ID NO: 204 - protein, 33 aa, Unknown
  Naturally occurring 2A or 2A-like self cleaving peptide
EARHKQKIVAPVKQTLNFDLLKLAGDVESNPGP

SEQ ID NO: 205 - protein, 7 aa, Tobacco etch virus
  VARIANT (2)..(2): Xaa = any amino acid
  VARIANT (3)..(3): Xaa = any amino acid
  VARIANT (5)..(5): Xaa = any amino acid
  VARIANT (7)..(7): Xaa is either Gly or Ser
EXXYXQX

SEQ ID NO: 206 - protein, 7 aa, Tobacco etch virus
ENLYFQG

SEQ ID NO: 207 - protein, 7 aa, Tabacco etch virus
ENLYFQS

SEQ ID NO: 208 - protein, 4 aa, Artificial Sequence
  Thrombin cleavable linker
GRGD

SEQ ID NO: 209 - protein, 6 aa, Artificial Sequence
  Thrombin cleavable linker
GRGDNP

SEQ ID NO: 210 - protein, 5 aa, Artificial Sequence
  Thrombin cleavable linker
GRGDS

SEQ ID NO: 211 - protein, 7 aa, Artificial Sequence
  Thrombin cleavable linker
GRGDSPK

SEQ ID NO: 212 - protein, 4 aa, Artificial Sequence
  Elastase cleavable linker
AAPV

SEQ ID NO: 213 - protein, 4 aa, Artificial Sequence
  Elastase cleavable linker
AAPL

SEQ ID NO: 214 - protein, 4 aa, Artificial Sequence
  Elastase cleavable linker
AAPF

SEQ ID NO: 215 - protein, 4 aa, Artificial Sequence
  Elastase cleavable linker
AAPA

SEQ ID NO: 216 - protein, 4 aa, Artificial Sequence
  Elastase cleavable linker
AYLV

SEQ ID NO: 217 - protein, 6 aa, Artificial Sequence
  Matrix metalloproteinase cleavable linker
  VARIANT (3)..(3): Xaa = Any amino acid
  VARIANT (6)..(6): Xaa = Any amino acid
GPXGPX

SEQ ID NO: 218 - protein, 4 aa, Artificial Sequence
  Matrix metalloproteinase cleavable linker
  VARIANT (4)..(4): Xaa = Any amino acid
LGPX

SEQ ID NO: 219 - protein, 6 aa, Artificial Sequence
  Matrix metalloproteinase cleavable linker
  VARIANT (6)..(6): Xaa = Any amino acid
GPIGPX

SEQ ID NO: 220 - protein, 5 aa, Artificial Sequence
  Matrix metalloproteinase cleavable linker
  VARIANT (5)..(5): Xaa = Any amino acid
APGLX

SEQ ID NO: 221 - protein, 7 aa, Artificial Sequence
  Collagenase cleavable linker
  VARIANT (7)..(7): Xaa = Any amino acid
PLGPDRX

SEQ ID NO: 222 - protein, 7 aa, Artificial Sequence
  Collagenase cleavable linker
  VARIANT (7)..(7): Xaa = Any amino acid
PLGLLGX

SEQ ID NO: 223 - protein, 7 aa, Artificial Sequence
  Collagenase cleavable linker
PQGIAGW

SEQ ID NO: 224 - protein, 5 aa, Artificial Sequence
  Collagenase cleavable linker
PLGCH

SEQ ID NO: 225 - protein, 6 aa, Artificial Sequence
  Collagenase cleavable linker
PLGLYA

SEQ ID NO: 226 - protein, 7 aa, Artificial Sequence
  Collagenase cleavable linker
PLALWAR

SEQ ID NO: 227 - protein, 7 aa, Artificial Sequence
  Collagenase cleavable linker
PLAYWAR

SEQ ID NO: 228 - protein, 7 aa, Artificial Sequence
  Stromelysin cleavable linker
PYAYYMR

SEQ ID NO: 229 - protein, 7 aa, Artificial Sequence
  Gelatinase cleavable linker
PLGMYSR

SEQ ID NO: 230 - protein, 4 aa, Artificial Sequence
  Angiotensin converting enzyme cleavable linker
GDKP

SEQ ID NO: 231 - protein, 5 aa, Artificial Sequence
  Angiotensin converting enzyme cleavable linker
GSDKP

SEQ ID NO: 232 - protein, 4 aa, Artificial Sequence
  Cathepsin B cleavable linker
ALAL

SEQ ID NO: 233 - protein, 4 aa, Artificial Sequence
  Cathepsin B cleavable linker
GFLG